European Patent Specification EP 3 364 997 B1, published January 17, 2024. Title: METHODS AND COMPOSITIONS FOR CORRECTING METABOLIC IMBALANCE IN NEURODEGENERATIVE DISEASE. Applicant: University of Massachusetts. Application Not Yet Assigned. The sequence listing filed with the application follows.

SEQUENCE LISTING (4 sequences)

SEQ ID NO: 1 - DNA, 948 bp, Artificial Sequence
  Synthetic Polynucleotide
gccaccatgacaagctgccacatcgccgaggagcacatccagaaagtcgccatttttgggggaactcacggtaacgaactcacaggggtcttcctggtgaagcactggctcgagaacggcgcagaaatccagagaaccggactggaggtgaaacccttcattacaaatcctcgggccgtcaagaaatgcactcgctacatcgactgtgatctgaaccggatttttgatctggaaaatctcggcaagaaaatgtccgaggacctgccatacgaagtgaggagagctcaggagatcaaccacctcttcggacccaaggacagcgaagattcctatgacatcatttttgatctgcataacaccacatcaaatatggggtgcaccctgatcctcgaggacagccgcaacaatttcctgatccagatgtttcactatattaagacaagtctggcaccactcccctgttacgtgtatctgattgagcatccctctctcaagtacgctactacccgaagtatcgcaaaatatcctgtggggattgaagtcggtcctcagccacagggagtcctgcgagccgatatcctcgaccagatgaggaagatgatcaaacatgctctggatttcattcaccacttcaacgagggcaaggagttccccccttgcgccatcgaggtgtacaagatcattgaaaaagtcgattatcctcgggacgagaacggcgaaattgccgctatcattcacccaaatctgcaggaccaggattggaagcccctccatcctggggatccaatgttcctgacactcgacggtaaaactatcccactgggcggagactgtaccgtgtaccccgtgtttgtcaatgaggcagcctactatgagaagaaagaagctttcgccaaaacaacaaaactcactctcaatgctaaatctattcggtgctgcctccactga

SEQ ID NO: 2 - protein, 313 aa, Artificial Sequence
  Synthetic Polypeptide
MTSCHIAEEHIQKVAIFGGTHGNELTGVFLVKHWLENGAEIQRTGLEVKPFITNPRAVKKCTRYIDCDLNRIFDLENLGKKMSEDLPYEVRRAQEINHLFGPKDSEDSYDIIFDLHNTTSNMGCTLILEDSRNNFLIQMFHYIKTSLAPLPCYVYLIEHPSLKYATTRSIAKYPVGIEVGPQPQGVLRADILDQMRKMIKHALDFIHHFNEGKEFPPCAIEVYKIIEKVDYPRDENGEIAAIIHPNLQDQDWKPLHPGDPMFLTLDGKTIPLGGDCTVYPVFVNEAAYYEKKEAFAKTTKLTLNAKSIRCCLH

SEQ ID NO: 3 - DNA, 915 bp, Artificial Sequence
  Synthetic Polynucleotide
gccaccatgcactgcgggccacctgatatggtctgtgaaactaagattgtcgctgccgaggatcacgaggctctgcctggagctaaaaaagatgctctgctggccgccgccggcgccatgtggccccctctgccagcagcaccaggaccagcagcagcaccacccgcccctccacccgcccctgtggcccagccacacggcggcgccggcggcgccggccctccaggcggccggggcgtgtgcatccgggagttcagagcagcagagcaggaggcagcaaggagaatcttttatgacggcatcatggagcggatccccaacaccgccttcaggggactgaggcagcaccctagagcacagctgctgtacgcactgctggccgccctgtgctttgccgtgagcaggtccctgctgctgacctgtctggtgcccgccgccctgctgggactgaggtactattacagccggaaagtgatcagagcctatctggagtgcgccctgcacacagacatggccgatatcgagcagtattacatgaagccccctggctcctgtttctgggtggccgtgctggacggaaacgtggtgggaatcgtggcagcaagggcacacgaggaggacaataccgtggagctgctgcgcatgtctgtggatagcaggttccgcggcaagggaatcgcaaaggccctgggaaggaaggtgctggagtttgccgtggtgcacaattactctgccgtggtgctgggcaccacagcagtgaaggtggcagcccacaagctgtatgagtccctgggctttaggcacatgggcgcctctgatcactacgtgctgcctggcatgacactgtccctggccgagagactgttcttccaggtccgctaccatagatatagactgcagctgagggaggagtga

SEQ ID NO: 4 - protein, 302 aa, Artificial Sequence
  Synthetic Polypeptide
MHCGPPDMVCETKIVAAEDHEALPGAKKDALLAAAGAMWPPLPAAPGPAAAPPAPPPAPVAQPHGGAGGAGPPGGRGVCIREFRAAEQEAARRIFYDGIMERIPNTAFRGLRQHPRAQLLYALLAALCFAVSRSLLLTCLVPAALLGLRYYYSRKVIRAYLECALHTDMADIEQYYMKPPGSCFWVAVLDGNVVGIVAARAHEEDNTVELLRMSVDSRFRGKGIAKALGRKVLEFAVVHNYSAVVLGTTAVKVAAHKLYESLGFRHMGASDHYVLPGMTLSLAERLFFQVRYHRYRLQLREE